European Patent Specification EP 3 662 910 B1, published September 18, 2024. Title: PHARMACOPHORE FOR TRAIL INDUCTION. Applicant: The Scripps Research Institute. The sequence listing filed with the application follows.

SEQUENCE LISTING (4 sequences)

SEQ ID NO: 1 - DNA, 22 bp, Artificial Sequence
  A synthetic primer
gacaccatttctacagttccag

SEQ ID NO: 2 - DNA, 22 bp, Artificial Sequence
  A synthetic primer
cggatagctggtgtacttgtag

SEQ ID NO: 3 - DNA, 22 bp, Artificial Sequence
  A synthetic primer
acagacctgcgtgctgatcgtg

SEQ ID NO: 4 - DNA, 21 bp, Artificial Sequence
  A synthetic primer
acgagctgacggagttgccac